European Patent Application EP 4 223 884 A1, published August 9, 2023. Title: A method for improving the stability of a composition containing flavin-dependent lactate dehydrogenase. Applicant: Kikkoman Corporation. The sequence listing filed with the application follows.

SEQUENCE LISTING (11 sequences)

SEQ ID NO: 1 - protein, 506 aa, enzyme
MNKQKISPAEVAKHNKPDDCWVVINGYVYDLTRFLPNHPGGQDVIKFNAGKDVTAIFEPLHAPNVIDKYIAPEKKLGPLQGSMPPELVCPPYAPGETKEDIARKEQLKSLLPPLDNIINLYDFEYLASQTLTKQAWAYYSSGANDEVTHRENHNAYHRIFFKPKILVDVRKVDISTDMLGSHVDVPFYVSATALCKLGNPLEGEKDVARGCGQGVTKVPQMISTLASCSPEEIIEAAPSDKQIQWYQLYVNSDRKITDDLVKNVEKLGVKALFVTVDAPSLGQREKDMKLKFSNTKAGPKAMKKTNVEESQGASRALSKFIDPSLTWKDIEELKKKTKLPIVIKGVQRTEDVIKAAEIGVSGVVLSNHGGRQLDFSRAPIEVLAETMPILEQRNLKDKLEVFVDGGVRRGTDVLKALCLGAKGVGLGRPFLYANSCYGRNGVEKAIEILRDEIEMSMRLLGVTSIAELKPDLLDLSTLKARTVGVPNDVLYNEVYEGPTLTEFEDA

SEQ ID NO: 2 - DNA, 1521 bp, enzyme
atgaacaaacagaaaatctccccggcggaagtggctaaacataacaaaccggatgactgctgggtggtgatcaacggctatgtgtacgatctgacccgttttctgccgaaccacccgggcggtcaggatgttatcaaattcaacgccggtaaagacgtcacggctatcttcgaaccgctgcatgcgccgaatgtgattgataaatatatcgccccggagaaaaaactgggcccgctgcagggttctatgccgccagaactggtttgcccgccgtacgcaccgggcgaaaccaaagaagatattgctcgcaaagaacaactgaaatcgctgctgccgccgctggataacatcatcaacctgtacgacttcgaatacctggcgagccagaccctgacgaaacaagcgtgggcctattacagctctggcgcgaacgatgaagtgacccatcgtgaaaaccacaatgcctatcatcgcattttctttaaaccgaaaatcctggtcgatgtgcgtaaagtggatatttccaccgacatgctgggttcacacgttgacgtcccgttctatgtttctgcaacggctctgtgcaaactgggcaatccgctggaaggtgaaaaagatgtggcccgcggctgtggtcagggcgtgaccaaagttccgcaaatgattagtacgctggccagttgttccccggaagaaattatcgaagcggccccgtctgataaacagattcaatggtatcagctgtacgttaacagtgaccgtaaaatcaccgatgacctggtcaaaaatgtggaaaaactgggcgtcaaagcactgtttgtgacggttgatgctccgtccctgggtcagcgcgaaaaagacatgaaactgaaattctcaaacaccaaagcaggcccgaaagctatgaagaaaaccaatgtggaagaatcacagggtgcgtcgcgtgccctgagcaaatttattgatccgagcctgacctggaaagacatcgaagaactgaaaaagaaaaccaaactgccgattgttatcaaaggtgtccagcgcaccgaagatgtcattaaagcagctgaaatcggcgtgtctggtgtggttctgagtaaccatggcggtcgtcagctggactttagccgcgcgccgattgaagttctggccgaaaccatgccgatcctggaacaacgtaatctgaaagataaactggaagtctttgtggatggcggtgtgcgtcgcggtaccgatgttctgaaagcgctgtgcctgggtgccaaaggtgtcggcctgggtcgtccgttcctgtatgcaaactcctgttacggccgcaatggtgtggaaaaagctattgaaatcctgcgtgatgaaattgaaatgtcgatgcgtctgctgggcgtgaccagcattgcagaactgaaaccggatctgctggacctgagtaccctgaaagcacgcacggttggtgtcccgaatgatgtcctgtataacgaagtgtatgaaggcccgaccctgacggaatttgaagatgcgtaa

SEQ ID NO: 3 - protein, 578 aa, enzyme
MLLRSLNSSARCVKQTTRTKVRYLSHVSGASMAKPTLKNNSRESNKSRNYLIAAVTALAVSTSIGVAVHVKDPLYNDATGSDSPRSISVDEFVKHNSQNDCWIAINGKVYDFTDFIPNHPGGVPPLVNHAGYDGTKLYEKLHPKGTIEKFLPKDKFLGVLDGEAPKLEADYLVDDDEQERLDYLNNLPPLSSIQNVYDFEYLAKKILPKDAWAYYSCGADDEITMRENHYAYQRVYFRPRICVDVKEVDTSYEMLGTKTSVPFYVSATALAKLGHPDGECSIARGAGKEGVVQMISTLSSMSLDEIAAARIPGATQWFQLYINEDRNVAKGLVKHAEDLGMKAIFITVDAPSLGNREKDKRLKFVNDTDVDLGDSADRNSGASKALSSFIDASVSWNDVKAVKSWTKLPVLVKGVQTVEDVIEAYDAGCQGVVLSNHGGRQLDTAPPPIELLAETVPTLKRLGKLRPDFEILIDGGVKRGTDILKAVAIGGQDVRVSVGMGRPFLYANSCYGEAGVRKLIQNLKDELEMDMRLLGVTKMDQLSSKHVDTKRLIGRDAINYLYDNVYSPIETVKFNNED

SEQ ID NO: 4 - protein, 502 aa, enzyme
MATGSDSPRSISVDEFVKHNSQNDCWIAINGKVYDFTDFIPNHPGGVPPLVNHAGYDGTKLYEKLHPKGTIEKFLPKDKFLGVLDGEAPKLEADYLVDDDEQERLDYLNNLPPLSSIQNVYDFEYLAKKILPKDAWAYYSCGADDEITMRENHYAYQRVYFRPRICVDVKEVDTSYEMLGTKTSVPFYVSATALAKLGHPDGECSIARGAGKEGVVQMISTLSSMSLDEIAAARIPGATQWFQLYINEDRNVAKGLVKHAEDLGMKAIFITVDAPSLGNREKDKRLKFVNDTDVDLGDSADRNSGASKALSSFIDASVSWNDVKAVKSWTKLPVLVKGVQTVEDVIEAYDAGCQGVVLSNHGGRQLDTAPPPIELLAETVPTLKRLGKLRPDFEILIDGGVKRGTDILKAVAIGGQDVRVSVGMGRPFLYANSCYGEAGVRKLIQNLKDELEMDMRLLGVTKMDQLSSKHVDTKRLIGRDAINYLYDNVYSPIETVKFNNED

SEQ ID NO: 5 - DNA, 1509 bp, enzyme
atggctactgggtcagatagtcctagaagcattagcgttgacgaattcgttaaacacaacagccagaatgattgttggattgccattaatggaaaagtttatgatttcacggatttcattcctaaccacccagggggtgtcccacccctggtgaatcacgccggttacgacggtacgaaactgtatgaaaaactgcatcctaaaggtaccattgaaaaatttttaccgaaagataaatttcttggcgtgttagacggcgaggctccgaagctggaggcggattacctggttgacgacgacgaacaggaaagactggactacttgaacaatttgccgcctttatccagtattcagaatgtctacgacttcgagtatttggcaaaaaagattctgcctaaggatgcttgggcctactacagctgcggtgcagatgacgagataacgatgcgcgaaaaccattatgcgtatcaacgcgtttacttccgtccgcgcatttgcgttgatgtgaaggaagttgatactagctatgaaatgctgggtactaaaaccagcgtgccgttttatgttagtgccaccgcattggcgaaactgggtcatcccgatggtgagtgctcaattgcacgtggcgctggtaaggaaggtgtcgttcagatgatttcaactctgtcatcaatgagtctggatgaaatagcggcggcacggattccaggggcgacccagtggtttcagctgtatattaatgaggatcgtaatgtcgctaagggtctggttaaacatgcagaagacctgggtatgaaggcaatttttataaccgtggacgcaccgtccttaggcaatcgtgagaaggataagcgtctgaaatttgttaacgacacggatgtagatctgggggactcagccgaccgtaattcgggagcgtccaaggctctgagttcgtttatagatgcaagtgtttcttggaacgatgtgaaagccgtgaagtcgtggaccaaattacccgtgctggttaaaggagttcagaccgtggaagatgtaatagaagcctatgatgcaggttgtcagggggtcgtactgtctaaccatggagggcgccaactggacactgccccaccaccgatcgaacttctggcagagacggtgccgacattgaaacgtttaggcaaattacgcccggattttgaaatcttaatcgatggcggcgtgaaacgtgggacagacatattaaaagccgtggcgatcggcggccaagatgtaagagtatctgtaggcatgggacgcccatttttatatgctaactcttgttatggagaggcgggagtccggaaattgatccaaaatttgaaagatgagcttgaaatggatatgcgccttcttggcgtcacaaaaatggatcaactttcttctaaacatgtagatacaaaacggcttatcggacgggatgctatcaactatctttatgataatgtatattcccctatcgaaacagtcaaatttaataatgaagattaa

SEQ ID NO: 6 - protein, 571 aa, enzyme
MIKNSFVKTTGCICKSHSTTLARKYQFRSLTTTSNVGKRYSNNGKNTIKFSFTFIIASALALVTTHKVTNDVTPKSKNIISVEDFVKHNSKDDCWIAINGKVFDVTEFIPDHPGGEIPLISHAGYDGTKVYEKIHPKGTIEKFLPEDKFLGILDGDAPKLEADYLIDDDEEERLKYIENIPPISNIQNSYDFEYIAKHILPKDAWAYYSCGSDDEISMRENHYAYQRVYFRPRICVNVKEVDTSTTLLGTPTSVPFYVSATALAKLGHPDGECSIARGAGKEGVIQMISTLSSNSLEEIAQARIPGATQWFQLYINENRETAKRMVKEAEDLGMKAIFITVDAPSLGNREKDKREKFVDDTDVDLGDGVDRNSGASKALSAFIDCSVDWNDVKEVKSWTKLPVLIKGVQTVEDVIEAYDAGCQGVVLSNHGGRQLDTAPPPIELLAETVPVMKKLNKLRPDFEILLDGGVKRGTDILKAVAIGGKDIRVGVGLGRPFLYANSCYGEDGVRKLIQILKDELEMDMRLLGVTKISDLTPKFVDTRRLIGREAVNYLYDDVYNHIPTVKFRNDD

SEQ ID NO: 7 - protein, 505 aa, enzyme
MVTNDVTPKSKNIISVEDFVKHNSKDDCWIAINGKVFDVTEFIPDHPGGEIPLISHAGYDGTKVYEKIHPKGTIEKFLPEDKFLGILDGDAPKLEADYLIDDDEEERLKYIENIPPISNIQNSYDFEYIAKHILPKDAWAYYSCGSDDEISMRENHYAYQRVYFRPRICVNVKEVDTSTTLLGTPTSVPFYVSATALAKLGHPDGECSIARGAGKEGVIQMISTLSSNSLEEIAQARIPGATQWFQLYINENRETAKRMVKEAEDLGMKAIFITVDAPSLGNREKDKREKFVDDTDVDLGDGVDRNSGASKALSAFIDCSVDWNDVKEVKSWTKLPVLIKGVQTVEDVIEAYDAGCQGVVLSNHGGRQLDTAPPPIELLAETVPVMKKLNKLRPDFEILLDGGVKRGTDILKAVAIGGKDIRVGVGLGRPFLYANSCYGEDGVRKLIQILKDELEMDMRLLGVTKISDLTPKFVDTRRLIGREAVNYLYDDVYNHIPTVKFRNDD

SEQ ID NO: 8 - DNA, 1518 bp, enzyme
atggtaacaaacgatgttacccctaagtcaaaaaatatcatttcagttgaagatttcgttaagcacaatagtaaagatgactgttggatcgcaataaacggtaaggtgtttgacgttacagaatttattcctgaccaccctggtggcgagattccgttgatcagccacgctggttacgatggtaccaaagtctacgagaaaattcatccgaaaggaaccatagagaagtttttaccggaagacaaattcctgggcatacttgacggtgacgcaccgaagctggaggcggactatctgatagacgacgatgaggaggagcgccttaagtatatagagaacatccctccgattagtaatatccaaaacagttatgattttgagtatatcgccaagcatattttgccaaaagacgcctgggcctactattcatgcggttcagacgacgaaatctcaatgcgcgagaatcattacgcatatcagcgcgtttattttcgcccgcgcatatgcgttaatgtgaaagaggttgacactagtacaacactgcttggaacacctacaagtgttccgttttatgtatctgcgaccgccctggctaagctgggtcatccggatggcgaatgttctatcgcccgtggcgccggtaaagaaggtgttattcagatgatatccaccttgtcttctaactctctggaggaaatcgcccaagccagaattccaggcgcaacccaatggtttcaactttatataaatgaaaatcgtgaaactgctaaacgcatggttaaagaagcggaagaccttgggatgaaagcgatattcatcaccgttgatgctccgtccctggggaaccgcgaaaaagacaaaagagaaaaattcgtggatgacactgatgtcgatttaggggacggagttgatcgtaacagcggcgcgagcaaggcactgagcgcgtttattgattgcagcgttgattggaatgatgtgaaagaagtaaagtcctggacgaaactgcctgtgttaattaaaggtgtgcagaccgtggaagatgtgatcgaagcgtacgatgctggctgtcagggtgtggtactgtccaatcatggcggtagacagctggatactgctccccccccaattgaactgcttgctgaaactgtccccgtgatgaagaaattaaacaaactgagacccgattttgaaattctgttagatggcggtgtcaaacgtggcacggatattctgaaagcggtagcaatcggaggcaaagatattcgtgtgggagtgggactggggcgtccatttctgtatgcaaattcgtgttatggggaagatggagtccgtaaactgattcagattttaaaagatgaacttgaaatggatatgcggttattaggggtcacgaaaatttcggatttgacgccaaaattcgtagatacgcgtcggttgattgggcgggaagcagtcaactatttgtacgatgatgtatacaatcatattccaacggtcaaattccggaatgatgattaa

SEQ ID NO: 9 - protein, 558 aa, enzyme
MWRTSYRAFTTGKKPLPRLSRTLASSAKRFPRRSLGAAIVAGLGAALVCTQLPGRPQLSSESPALPKRIVPVAEFVKHNRPDDCWVAIRGQVYDMTEFLPHHPGGQSPIIRYSGHDATELFEQLHPKGTIEKHLPKEKHLGQLDGPAPTLEVAEDEFEEERLENVANMPNVNEVMNLHDFEYIAKKILPKGAWAYYSSGADDEVSMRENHYAYQRIYFRPRVLVDVSKVDTSTTLLGTPTSVPFYVSATALAKLGHPDGECSIARGAGKEGVIQMISTLASNSLEEIAAARVPGATQWFQLYVNEDRNVAFEMVKKAEKLGIKAIFVTVDAPSLGNREKDARVKFEGESDVQKSNEVVRSQGASRALSSFIDTRLTWDDVKKIKQSTKLPVLIKGVQRLEDVVQAVDDGFDGVVLSNHGGRQLDTAPPPVELLAEVVPELKRRNKLRPDFEIFIDGGVRRGTDILKALALGGQNVRVGVGLGRPFLYANSSYGENGVRKAIQLLKDELEMDMRLLGVRNLRELDETFVDTRRLIGRDAPDELYNQLYSPLKTVKFRNE

SEQ ID NO: 10 - protein, 503 aa, enzyme
MQLSSESPALPKRIVPVAEFVKHNRPDDCWVAIRGQVYDMTEFLPHHPGGQSPIIRYSGHDATELFEQLHPKGTIEKHLPKEKHLGQLDGPAPTLEVAEDEFEEERLENVANMPNVNEVMNLHDFEYIAKKILPKGAWAYYSSGADDEVSMRENHYAYQRIYFRPRVLVDVSKVDTSTTLLGTPTSVPFYVSATALAKLGHPDGECSIARGAGKEGVIQMISTLASNSLEEIAAARVPGATQWFQLYVNEDRNVAFEMVKKAEKLGIKAIFVTVDAPSLGNREKDARVKFEGESDVQKSNEVVRSQGASRALSSFIDTRLTWDDVKKIKQSTKLPVLIKGVQRLEDVVQAVDDGFDGVVLSNHGGRQLDTAPPPVELLAEVVPELKRRNKLRPDFEIFIDGGVRRGTDILKALALGGQNVRVGVGLGRPFLYANSSYGENGVRKAIQLLKDELEMDMRLLGVRNLRELDETFVDTRRLIGRDAPDELYNQLYSPLKTVKFRNE

SEQ ID NO: 11 - DNA, 1512 bp, enzyme
atgcaactttcttcagagagtccagctctgcccaaacggattgttcccgtagcagagttcgtcaagcataatcgtcccgatgactgctgggttgcgatacggggtcaggtttatgatatgacggagttcctgccgcaccatcctggcggtcagagccctattatacgttattcaggccacgatgcaacggagcttttcgaacaattgcatcctaagggtacaattgaaaagcatttaccgaaagagaagcatttgggccaactggatggtccggcccctaccctggaagtcgccgaagacgaattcgaagaagaacgtctggagaatgtagctaatatgcctaatgttaatgaagttatgaacttgcatgattttgagtatatagcaaagaagattctgccgaagggtgcctgggcgtattatagcagtggtgctgatgacgaggttagcatgcgtgaaaatcactatgcctaccaacgcatttattttcgtccgagagttttagttgatgttagcaaagttgatacgagcactacccttttgggtacgcccacaagtgttcctttttatgtttcggccaccgctttagcaaagcttggccacccggacggtgaatgtagcatagcacggggcgccggtaaagagggtgtgatacagatgatttctaccctggcatctaattcgctggaagaaattgccgcggcacgggttccgggtgcaacgcaatggttccagctgtacgtcaatgaagatcgcaatgtggctttcgaaatggttaaaaaagctgagaagttaggcattaaagcgattttcgtaactgtggatgcaccgtcactgggcaaccgtgaaaaagacgctcgtgttaaatttgaaggtgagtcagatgtgcaaaaatcaaacgaggtggtacggagtcagggtgcgagtcgcgcgctgtcttcgtttatcgacacacgtttaacctgggatgatgtgaaaaaaatcaaacagtctactaaactgccagtgttaattaaaggcgtacagcgtctggaagacgtcgtacaggcagtagatgacggatttgatggggtggtgctgtccaaccatggcgggcggcagctggataccgcaccgcctccggtcgaacttctggctgaggtggtgccggaactgaaacgtcgtaataaactgcgtccagactttgagatctttatcgacggaggcgtccgcagagggactgacatcctgaaagcgttagcgctgggcggacagaacgtacgcgtcggagtggggctggggcgcccatttctgtatgccaattcctcctacggagagaatggggtgagaaaagccatccagttgttaaaagatgaacttgaaatggatatgcgcttgttaggagtgagaaacttacgcgaattggatgaaacctttgtcgatacacgccgcttgatcggacgcgatgcgccagatgaactttacaaccagctttactccccacttaaaacagtcaaatttagaaacgaataa